European Patent Application EP 4 296 372 A1, published December 27, 2023. Title: METHOD TO DETECT AND DISCRIMINATE CYTOSINE MODIFICATIONS. Applicant: UNIVERSITAT POMPEU FABRA (UPF). The sequence listing filed with the application follows.

SEQUENCE LISTING (6 sequences)

SEQ ID NO: 1 - DNA, 33 bp, Artificial Sequence
  first adapter oligonucleotide sequence (5´'3´)
  primer_bind (1)..(33): first adapter oligonucleotide sequence (5´'3´)
acactctttccctacacgacgctcttccgatct

SEQ ID NO: 2 - DNA, 34 bp, Artificial Sequence
  second adapter oligonucleotide sequence (5´'3´)
  primer_bind (1)..(34): second adapter oligonucleotide sequence (5´'3´)
agatcggaagagcacacgtctgaactccagtcac

SEQ ID NO: 3 - DNA, 40 bp, Artificial Sequence
  first splint oligonucleotide sequence (5´'3´)
  N_region (1)..(7): N" is a nucleotide selected from the group consisting of A, C, T, G. A random combination of 7 "N"
  misc_feature (1)..(7): n is a, c, g, or t
  misc_feature (8)..(40): first adapter oligonucleotide hybridization region
nnnnnnnagatcggaagagcgtcgtgtagggaaagagtgt

SEQ ID NO: 4 - DNA, 41 bp, Artificial Sequence
  second splint oligonucleotide sequence (5´'3´)
  misc_feature (1)..(34): second adapter oligonucleotide hybridization region
  N_region (35)..(41): N" is a nucleotide selected from the group consisting of A, C, T, G. It is a random sequence
  misc_feature (35)..(41): n is a, c, g, or t
gtgactggagttcagacgtgtgctcttccgatctnnnnnnn

SEQ ID NO: 5 - DNA, 62 bp, Artificial Sequence
  P5 Index primer
  N_region (29)..(36): N" is a nucleotide selected from the group consisting of A, C, T, G. This region is termed "index".
  misc_feature (30)..(36): n is a, c, g, or t
aatgatacggcgaccaccgagatctacacnnnnnnnacactctttccctacacgacgctctt

SEQ ID NO: 6 - DNA, 52 bp, Artificial Sequence
  P7 Index primer
  N_region (25)..(31): "N" is a nucleotide selected from the group consisting of A, C, T, G. This region is termed "index".
  misc_feature (25)..(31): n is a, c, g, or t
caagcagaagacggcatacgagatnnnnnnngtgactggagttcagacgtgt